European Patent Application EP 4 253 562 A2, published October 4, 2023. Title: DNA SEQUENCING USING HYDROGEL BEADS. Applicant: Illumina Inc. Application EP 22178045.5. The sequence listing filed with the application follows.

SEQUENCE LISTING (4 sequences)

SEQ ID NO: 1 - DNA, 20 bp, synthetic construct
  misc_feature 1..20: note = Synthetic Oligonucleotide
  source 1..20: mol_type = other DNA
aatgatacggcgaccaccga

SEQ ID NO: 2 - DNA, 21 bp, synthetic construct
  misc_feature 1..21: note = Synthetic Oligonucleotide
  source 1..21: mol_type = other DNA
caagcagaagacggcatacga

SEQ ID NO: 3 - DNA, 30 bp, synthetic construct
  misc_feature 1..30: note = Synthetic Oligonucleotide
  source 1..30: mol_type = other DNA
ttttttttttaatgatacggcgaccaccga

SEQ ID NO: 4 - DNA, 31 bp, synthetic construct
  misc_feature 1..31: note = Synthetic Oligonucleotide
  source 1..31: mol_type = other DNA
ttttttttttcaagcagaagacggcatacga